European Patent Specification EP 3 792 357 B1, published May 7, 2025. Title: Predetermined nucleotide substitutions. Applicant: Carlsberg A/S. The sequence listing filed with the application follows.

SEQUENCE LISTING (26 sequences)

SEQ ID NO: 1 - DNA, 1089 bp, Hordeum vulgare
atgtctcggctcgccgaccttctcagcctcgacctgtccggctgcaccggcaagatcatcgccgagtacatatgggtcggcggcaccgggatggacgtcaggagcaaagccaggacgcttcccggacccgtggacgaccccagcaagcttccaaagtggaatttcgacggctccagcaccggccaagccacgggcgacgacagcgaagtcatcctccgaccccaagccatcttcagggacccgttcaggaaagggaacaacatcctggtcatctgtgactgctatgcgcctaccggagagccgattccgagcaacaagcggtacaacgcggcgaggatattcggccatcctgatgtcaagtctgaagaaccatggtatgggattgagcaggagtacacccttctccagaaggacaccaactggcccattggctggccactagggggttaccctggccctcaggggccttactactgcgccgcgggtgcggagaaatcttacgggcgcgacatcgtcgacgcccactacaaggcctgcctctacgccggcatcaacatcggcggcatcaatgcagaagtcatgccagggcagtgggagttccaagtcggcccttccgtcggyatctccgccggcgacgagctctgggcggctcgctacattctcgagaggatcactgagatcgccggcgtcgtcgtctccttcgaccccaaaccgatcccgggagagtggaacggtgccggtgcccacacaaactacagcaccaagtcgatgaggagcgagggcgggtacgaggtgatcaagagggcgatcaagaagctcgaggcgcggcacacggagcacatagccgcctacggggaaggcaacgagcgccggctcaccggccgccacgagaccgccgacatcaacaccttcgtatggggcgtggcaaaccgcggcgcgtcggtgcgggtggggcgcgacaccgagaaggaaggcaggggctacttcgaggaccggaggccggcgtccaacatggatccctacgtcgtcacctccatgatcgccgagaccaccatcctctggaaggccggtctctccaatggcaagtag

SEQ ID NO: 2 - protein, 362 aa, Hordeum vulgare
MSRLADLLSLDLSGCTGKIIAEYIWVGGTGMDVRSKARTLPGPVDDPSKLPKWNFDGSSTGQATGDDSEVILRPQAIFRDPFRKGNNILVICDCYAPTGEPIPSNKRYNAARIFGHPDVKSEEPWYGIEQEYTLLQKDTNWPIGWPLGGYPGPQGPYYCAAGAEKSYGRDIVDAHYKACLYAGINIGGINAEVMPGQWEFQVGPSVGISAGDELWAARYILERITEIAGVVVSFDPKPIPGEWNGAGAHTNYSTKSMRSEGGYEVIKRAIKKLEARHTEHIAAYGEGNERRLTGRHETADINTFVWGVANRGASVRVGRDTEKEGRGYFEDRRPASNMDPYVVTSMIAETTILWKAGLSNGK

SEQ ID NO: 3 - DNA, 20 bp, Artificial sequence
  Primer
gtgatcaagagggcgatcaa

SEQ ID NO: 4 - DNA, 20 bp, Artificial sequence
  Primer
caagtctcaactcgccgtat

SEQ ID NO: 5 - DNA, 14 bp, Artificial sequence
  Probe
aagacaacgagcgc

SEQ ID NO: 6 - DNA, 14 bp, Artificial sequence
  Probe
aaggcaacgagcgc

SEQ ID NO: 7 - protein, 503 aa, Saccharomyces cerevisiae
MRKLNPALEFRDFIQVLKDEDDLIEITEEIDPNLEVGAIMRKAYESHLPAPLFKNLKGASKDLFSILGCPAGLRSKEKGDHGRIAHHLGLDPKTTIKEIIDYLLECKEKEPLPPITVPVSSAPCKTHILSEEKIHLQSLPTPYLHVSDGGKYLQTYGMWILQTPDKKWTNWSIARGMVVDDKHITGLVIKPQHIRQIADSWAAIGKANEIPFALCFGVPPAAILVSSMPIPEGVSESDYVGAILGESVPVVKCETNDLMVPATSEMVFEGTLSLTDTHLEGPFGEMHGYVFKSQGHPCPLYTVKAMSYRDNAILPVSNPGLCTDETHTLIGSLVATEAKELAIESGLPILDAFMPYEAQALWLILKVDLKGLQALKTTPEEFCKKVGDIYFRTKVGFIVHEIILVADDIDIFNFKEVIWAYVTRHTPVADQMAFDDVTSFPLAPFVSQSSRSKTMKGGKCVTNCIFRQQYERSFDYITCNFEKGYPKGLVDKVNENWKRYGYK

SEQ ID NO: 8 - protein, 101 aa, Triticum aestivum
MAKISFLLVALLVLAVGFPVEVMGGGGGGGGGGGGGNLKPWECSSKCSSRCSGTQYKKACLTYCNKCCATCLCVPPGTYGNKGACPCYNNWKTKEGGPKCP

SEQ ID NO: 9 - DNA, 15 bp, Artificial sequence
  Primer
cgcctgcccctgcta

SEQ ID NO: 10 - DNA, 31 bp, Artificial sequence
  Primer
agaagaagaagaagaagaagaaaaccaagaa

SEQ ID NO: 11 - DNA, 17 bp, Artificial sequence
  Probe
caacaactgaaagacca

SEQ ID NO: 12 - DNA, 17 bp, Artificial sequence
  Probe
caacaactggaagacca

SEQ ID NO: 13 - DNA, 17 bp, Artificial sequence
  Primer
catgtttcagacggtgg

SEQ ID NO: 14 - DNA, 20 bp, Artificial sequence
  Primer
catacctctagcaattgacc

SEQ ID NO: 15 - DNA, 20 bp, Artificial sequence
  Probe
acgtacggaatgtagattct

SEQ ID NO: 16 - DNA, 18 bp, Artificial sequence
  Probe
acgtacggaatgtggatt

SEQ ID NO: 17 - DNA, 1260 bp, Hordeum vulgare
atggcgtcgtcgagcttcaaggtgacgcggatctcggagggcgcggtgaagccggcgtcggagacgcccgaccacacgctgccgctggcgtgggtggaccggtacccgacccaccgcggcctggtggagtcgatgcacatcttccggtccggcgccgacgcggcccccggcgtgatccgcgaggcgctgggcaaggcgctggccttcttctacccgctggcggggcgcatcgtggagcagccggagaaggggtgccccgccatccgctgcaccgccgacggcgtctacttcgcggaggccgtcgccgagtgcagcctggaggacgtccggttcctggagcgccccctgctgctccccaaggaggacctcgtcccctaccccgccgccgatctctgggccgtcgagccccacaacaccatcatgatgatgcagatcacgaaattcacatgcggcgggttcgtgatgggcctccggttcaaccacgcgtcggcggacggcatgggcgcggcgcagttcatcaaggcggtcggcgacatggcccgggggctcccggagccgacggtgaagccggtgtgggacagggagaagttccccaacccgagcatcaagccgggccctctcccggagctcccggtgctggcgctggactacatcgtgctcgacttccccacgggctacatcgacgggctcaagacgcagtacaaggcgcacagcggcaagttctgctccggcttcgacgtgctgacggccaagctgtggcagtgccgtacccgggcgctgaacctggagccggacgccacggtgaagctgtgcttcttcgccagcgtgcgccacctgctgaagctggacgccgggtactacggcaactccatcttccccgtgaagatgtccgggacgagcaagaaggtgctggagtcgtcggtgatggaggtgatcgacatgatccgggaggccaagcagcggatggcggtggagttcttccagttcgccaaggaggagacgcggcaggaccccttccagatgaccttcgactacgagtccatctacgtctccgactggagcaagctggggttctccgacgtggactacggcttcggcccgcccatgttcgccggaccgctcgtcaacaacgacttcatcgcctccgtcgtcatcctcaaggcgccgctgccgctggacggcaccaggatgctcgccagctgcgtcaccaaggagcactcgcaggagttcgcccgcggcatgaaggaggacctgccatga

SEQ ID NO: 18 - DNA, 1260 bp, Artificial sequence
  Mutant cDNA
atggcgtcgtcgagcttcaaggtgacgcggatctcggagggcgcggtgaagccggcgtcggagacgcccgaccacacgctgccgctggcgtgagtggaccggtacccgacccaccgcggcctggtggagtcgatgcacatcttccggtccggcgccgacgcggcccccggcgtgatccgcgaggcgctgggcaaggcgctggccttcttctacccgctggcggggcgcatcgtggagcagccggagaaggggtgccccgccatccgctgcaccgccgacggcgtctacttcgcggaggccgtcgccgagtgcagcctggaggacgtccggttcctggagcgccccctgctgctccccaaggaggacctcgtcccctaccccgccgccgatctctgggccgtcgagccccacaacaccatcatgatgatgcagatcacgaaattcacatgcggcgggttcgtgatgggcctccggttcaaccacgcgtcggcggacggcatgggcgcggcgcagttcatcaaggcggtcggcgacatggcccgggggctcccggagccgacggtgaagccggtgtgggacagggagaagttccccaacccgagcatcaagccgggccctctcccggagctcccggtgctggcgctggactacatcgtgctcgacttccccacgggctacatcgacgggctcaagacgcagtacaaggcgcacagcggcaagttctgctccggcttcgacgtgctgacggccaagctgtggcagtgccgtacccgggcgctgaacctggagccggacgccacggtgaagctgtgcttcttcgccagcgtgcgccacctgctgaagctggacgccgggtactacggcaactccatcttccccgtgaagatgtccgggacgagcaagaaggtgctggagtcgtcggtgatggaggtgatcgacatgatccgggaggccaagcagcggatggcggtggagttcttccagttcgccaaggaggagacgcggcaggaccccttccagatgaccttcgactacgagtccatctacgtctccgactggagcaagctggggttctccgacgtggactacggcttcggcccgcccatgttcgccggaccgctcgtcaacaacgacttcatcgcctccgtcgtcatcctcaaggcgccgctgccgctggacggcaccaggatgctcgccagctgcgtcaccaaggagcactcgcaggagttcgcccgcggcatgaaggaggacctgccatga

SEQ ID NO: 19 - protein, 419 aa, Hordeum vulgare
MASSSFKVTRISEGAVKPASETPDHTLPLAWVDRYPTHRGLVESMHIFRSGADAAPGVIREALGKALAFFYPLAGRIVEQPEKGCPAIRCTADGVYFAEAVAECSLEDVRFLERPLLLPKEDLVPYPAADLWAVEPHNTIMMMQITKFTCGGFVMGLRFNHASADGMGAAQFIKAVGDMARGLPEPTVKPVWDREKFPNPSIKPGPLPELPVLALDYIVLDFPTGYIDGLKTQYKAHSGKFCSGFDVLTAKLWQCRTRALNLEPDATVKLCFFASVRHLLKLDAGYYGNSIFPVKMSGTSKKVLESSVMEVIDMIREAKQRMAVEFFQFAKEETRQDPFQMTFDYESIYVSDWSKLGFSDVDYGFGPPMFAGPLVNNDFIASVVILKAPLPLDGTRMLASCVTKEHSQEFARGMKEDLP

SEQ ID NO: 20 - DNA, 13 bp, Artificial sequence
  Primer
cccgaccacacgc

SEQ ID NO: 21 - DNA, 14 bp, Artificial sequence
  Primer
actccaccaggccg

SEQ ID NO: 22 - DNA, 15 bp, Artificial sequence
  Probe
ctggcgtgagtggac

SEQ ID NO: 23 - DNA, 14 bp, Artificial sequence
  Probe
ctggcgtgggtgga

SEQ ID NO: 24 - DNA, 14 bp, Artificial sequence
  Probe
ctggcgtgggtgga

SEQ ID NO: 25 - DNA, 306 bp, Triticum aestivum
atggccaagatctccttcctcctcgtggcgctcctcgtcctcgccgtcgggttccccgtggaggtgatgggaggtgggggcggcggcggcggtggcggtggcggcggcaacctcaagccatgggagtgctcgtccaagtgctcgtcgcggtgctcggggacgcagtacaagaaggcgtgcctgacctactgcaacaagtgctgcgccacctgcctctgcgtgccgccgggcacctacggcaacaagggcgcctgcccctgctacaacaactggaagaccaaggagggaggccccaagtgcccctag

SEQ ID NO: 26 - DNA, 1512 bp, Saccharomyces cerevisiae
atgaggaagctaaatccagctttagaatttagagactttatccaggtcttaaaagatgaagatgacttaatcgaaattaccgaagagattgatccaaatctcgaagtaggtgcaattatgaggaaggcctatgaatcccacttaccagccccgttatttaaaaatctcaaaggtgcttcgaaggatcttttcagcattttaggttgcccagccggtttgagaagtaaggagaaaggagatcatggtagaattgcccatcatctggggctcgacccaaaaacaactatcaaggaaatcatagattatttgctggagtgtaaggagaaggaacctctccccccaatcactgttcctgtgtcatctgcaccttgtaaaacacatatactttctgaagaaaaaatacatctacaaagcctgccaacaccatatctacatgtttcagacggtggcaagtacttacaaacgtacggaatgtggattcttcaaactccagataaaaaatggactaattggtcaattgctagaggtatggttgtagatgacaagcatatcactggtctggtaattaaaccacaacatattagacaaattgctgactcttgggcagcaattggaaaagcaaatgaaattcctttcgcgttatgttttggcgttcccccagcagctattttagttagttccatgccaattcctgaaggtgtttctgaatcggattatgttggcgcaatcttgggtgagtcggttccagtagtaaaatgtgagaccaacgatttaatggttcctgcaacgagtgagatggtatttgagggtactttgtccttaacagatacacatctggaaggcccatttggtgagatgcatggatatgttttcaaaagccaaggtcatccttgtccattgtacactgtcaaggctatgagttacagagacaatgctattctacctgtttcgaaccccggtctttgtacggatgagacacataccttgattggttcactagtggctactgaggccaaggagctggctattgaatctggcttgccaattctggatgcctttatgccttatgaggctcaggctctttggcttatcttaaaggtggatttgaaagggctgcaagcattgaagacaacgcctgaagaattttgtaagaaggtaggtgatatttactttaggacaaaagttggttttatagtccatgaaataattttggtggcagatgatatcgacatatttaacttcaaagaagtcatctgggcctacgttacaagacatacacctgttgcagatcagatggcttttgatgatgtcacttcttttcctttggctccctttgtttcgcagtcatccagaagtaagactatgaaaggtggaaagtgcgttactaattgcatatttagacagcaatatgagcgcagttttgactacataacttgtaattttgaaaagggatatccaaaaggattagttgacaaagtaaatgaaaattggaaaaggtacggatataaataa